European Patent Specification EP 3 934 428 B1, published May 8, 2024. Title: Bacillus halosaccharovorans strain, composition comprising the same, and uses thereof. Applicant: Futureco Bioscience SA. The sequence listing filed with the application follows.

SEQUENCE LISTING (7 sequences)

SEQ ID NO: 1 - DNA, 20 bp, Artificial Sequence
  Primer
agagtttgatcctggctcag

SEQ ID NO: 2 - DNA, 15 bp, Artificial Sequence
  Primer
accttgttacgactt

SEQ ID NO: 3 - DNA, 965 bp, Artificial Sequence
  Amplicon
  misc_feature (130)..(130): n is a, c, g, or t
  misc_feature (145)..(146): n is a, c, g, or t
tgcaagtcgagcgaatctgagggagcttgctcccaaagattagcggcggacgggtgagtaacacgtgggtaacctgcctgtaagattgggataactccgggaaaccggagctaataccggataacatttngaaccgcatggttcnnaattgaaagacggcttttagctgtcacttacagatggacccgcggcgcattagctagttggtgaggtaacggctcaccaaggcaacgatgcgtagccgacctgagagggtgatcggccacactgggactgagacacggcccagactcctacgggaggcagcagtagggaatcttccgcaatggacgaaagtctgacggagcaacgccgcgtgaacgatgaaggccttcgggtcgtaaagttctgttgttagggaagaacaagtaccagagtaactgctggtaccttgacggtacctaaccagaaagccacggctaactacgtgccagcagccgcggtaatacgtaggtggcaagcgttgtccggaattattgggcgtaaagcgcgcgcaggcggtttcttaagtctgatgtgaaagcccacggctcaaccgtggagggtcattggaaactggggaacttgagtgcagaagaggagagtggaattccacgtgtagcggtgaaatgcgtagagatgtggaggaacaccagtggcgaaggcgactctctggtctgtaactgacgctgaggcgcgaaagcgtggggagcgaacaggattagataccctggtagtccacgccgtaaacgatgagtgctaagtgttagagggtttccgccctttagtgctgcagcaaacgcattaagcactccgcctggggagtacggtcgcaagactgaaactcaaaggaattgacgggggcccgcacaagcggtggagcatgtggtttaattcgaagcaacgcgaagaaccttaccaggtcttgacatccttcgctacttcta

SEQ ID NO: 4 - DNA, 20 bp, Artificial Sequence
  Primer
cggaatcgctagtaatcgcg

SEQ ID NO: 5 - DNA, 20 bp, Artificial Sequence
  Primer
cccaatcatctgtcccacct

SEQ ID NO: 6 - DNA, 20 bp, Artificial Sequence
  Primer
tcgggtcgtaaagctctgtt

SEQ ID NO: 7 - DNA, 20 bp, Artificial Sequence
  Primer
ttctgcactcaagttcccca